European Patent Specification EP 3 700 937 B1, published July 15, 2026. Title: DPP3 binder directed to and binding to specific DPP3-epitopes and its use in the prevention and treatment of diseases / acute conditions that are associated with oxidative stress. Applicant: Sphingotec Therapeutics GmbH. The sequence listing filed with the application follows.

SEQUENCE LISTING (13 sequences)

SEQ ID NO: 1 - protein, 737 aa, Homo sapiens
MADTQYILPNDIGVSSLDCREAFRLLSPTERLYAYHLSRAAWYGGLAVLLQTSPEAPYIYALLSRLFRAQDPDQLRQHALAEGLTEEEYQAFLVYAAGVYSNMGNYKSFGDTKFVPNLPKEKLERVILGSEAAQQHPEEVRGLWQTCGELMFSLEPRLRHLGLGKEGITTYFSGNCTMEDAKLAQDFLDSQNLSAYNTRLFKEVDGEGKPYYEVRLASVLGSEPSLDSEVTSKLKSYEFRGSPFQVTRGDYAPILQKVVEQLEKAKAYAANSHQGQMLAQYIESFTQGSIEAHKRGSRFWIQDKGPIVESYIGFIESYRDPFGSRGEFEGFVAVVNKAMSAKFERLVASAEQLLKELPWPPTFEKDKFLTPDFTSLDVLTFAGSGIPAGINIPNYDDLRQTEGFKNVSLGNVLAVAYATQREKLTFLEEDDKDLYILWKGPSFDVQVGLHELLGHGSGKLFVQDEKGAFNFDQETVINPETGEQIQSWYRSGETWDSKFSTIASSYEECRAESVGLYLCLHPQVLEIFGFEGADAEDVIYVNWLNMVRAGLLALEFYTPEAFNWRQAHMQARFVILRVLLEAGEGLVTITPTTGSDGRPDARVRLDRSKIRSVGKPALERFLRRLQVLKSTGDVAGGRALYEGYATVTDAPPECFLTLRDTVLLRKESRKLIVQPNTRLEGSDVQLLEYEASAAGLIRSFSERFPEDGPELEEILTQLATADARFWKGPSEAPSGQA

SEQ ID NO: 2 - protein, 21 aa, Homo sapiens
CETVINPETGEQIQSWYRSGE

SEQ ID NO: 3 - protein, 6 aa, Homo sapiens
INPETG

SEQ ID NO: 4 - protein, 4 aa, Homo sapiens
ETGE

SEQ ID NO: 5 - protein, 116 aa, Mus musculus
QVTLKESGPGILQPSQTLSLTCSFSGFSLSTSGMSVGWIRQPSGKGLEWLAHIWWNDNKSYNPALKSRLTISRDTSNNQVFLKIASVVTADTGTYFCARNYSYDYWGQGTTLTVSS

SEQ ID NO: 6 - protein, 112 aa, Mus musculus
DVVVTQTPLSLSVSLGDPASISCRSSRSLVHSIGSTYLHWYLQKPGQSPKLLIYKVSNRFSGVPDRFSGSGSGTDFTLKISRVEAEDLGVYFCSQSTHVPWTFGGGTKLEIK

SEQ ID NO: 7 - protein, 10 aa, Mus musculus
GFSLSTSGMS

SEQ ID NO: 8 - protein, 7 aa, Mus musculus
IWWNDNK

SEQ ID NO: 9 - protein, 8 aa, Mus musculus
ARNYSYDY

SEQ ID NO: 10 - protein, 11 aa, Mus musculus
RSLVHSIGSTY

SEQ ID NO: 11 - protein, 9 aa, Mus musculus
SQSTHVPWT

SEQ ID NO: 12 - protein, 469 aa, Mus musculus
MDPKGSLSWRILLFLSLAFELSYGQITLKESGPTLVKPTQTLTLTCTFSGFSLSTSGMSVGWIRQPPGKALEWLAHIWWNDNKSYNPALKSRLTITRDTSKNQVVLTMTNMDPVDTGTYYCARNYSYDYWGQGTLVTVSSASTKGPSVFPLAPSSKSTSGGTAALGCLVKDYFPEPVTVSWNSGALTSGVHTFPAVLQSSGLYSLSSVVTVPSSSLGTQTYICNVNHKPSNTKVDKKVEPKSCDKTHTCPPCPAPELLGGPSVFLFPPKPKDTLMISRTPEVTCVVVDVSHEDPEVKFNWYVDGVEVHNAKTKPREEQYNSTYRVVSVLTVLHQDWLNGKEYKCKVSNKALPAPIEKTISKAKGQPREPQVYTLPPSRDELTKNQVSLTCLVKGFYPSDIAVEWESNGQPENNYKTTPPVLDSDGSFFLYSKLTVDKSRWQQGNVFSCSVMHEALHNHYTQKSLSLSPG

SEQ ID NO: 13 - protein, 239 aa, Mus musculus
METDTLLLWVLLLWVPGSTGDIVMTQTPLSLSVTPGQPASISCKSSRSLVHSIGSTYLYWYLQKPGQSPQLLIYKVSNRFSGVPDRFSGSGSGTDFTLKISRVEAEDVGVYYCSQSTHVPWTFGGGTKVEIKRTVAAPSVFIFPPSDEQLKSGTASVVCLLNNFYPREAKVQWKVDNALQSGNSQESVTEQDSKDSTYSLSSTLTLSKADYEKHKVYACEVTHQGLSSPVTKSFNRGEC